European Patent Application EP 4 578 873 A1, published July 2, 2025. Title: ANTI-HUMAN INTERLEUKIN 36 RECEPTOR MONOCLONAL ANTIBODY AND USE THEREOF. Applicant: Qyuns Therapeutics Co., Ltd. The sequence listing filed with the application follows.

SEQUENCE LISTING (11 sequences)

SEQ ID NO: 1 - protein, 5 aa, synthetic construct
NYAMG

SEQ ID NO: 2 - protein, 16 aa, synthetic construct
YISGGGSAYYASWAKG

SEQ ID NO: 3 - protein, 12 aa, synthetic construct
WAIKSYFFGMDL

SEQ ID NO: 4 - protein, 11 aa, synthetic construct
QASEYISSYLA

SEQ ID NO: 5 - protein, 7 aa, synthetic construct
QASTLAS

SEQ ID NO: 6 - protein, 12 aa, synthetic construct
QTNNAIHTYGGA

SEQ ID NO: 7 - protein, 120 aa, synthetic construct
EVQLVESGGGLVQPGGSLRLSCAASGIDLSNYAMGWVRQAPGKGLEWVGYISGGGSAYYASWAKGRFTISRDNSKNTLYLQMNSLRAEDTAVYYCARWAIKSYFFGMDLWGQGTLVTVSS

SEQ ID NO: 8 - protein, 110 aa, synthetic construct
DIQMTQSPSSVSASVGDRVTITCQASEYISSYLAWYQQKPGKAPKLLIYQASTLASGVPSRFSGSGSGTDFTLTISSLQPEDFATYYCQTNNAIHTYGGAFGGGTKVEIK

SEQ ID NO: 9 - protein, 335 aa, synthetic construct
MWSLLLCGLSIALPLSVTADGCKDIFMKNEILSASQPFAFNCTFPPITSGEVSVTWYKNSSKIPVSKIIQSRIHQDETWILFLPMEWGDSGVYQCVIKGRDSCHRIHVNLTVFEKHWCDTSIGGLPNLSDEYKQILHLGKDDSLTCHLHFPKSCVLGPIKWYKDCNEIKGERFTVLETRLLVSNVSAEDRGNYACQAILTHSGKQYEVLNGITVSITERAGYGGSVPKIIYPKNHSIEVQLGTTLIVDCNVTDTKDNTNLRCWRVNNTLVDDYYDESKRIREGVETHVSFREHNLYTVNITFLEVKMEDYGLPFMCHAGVSTAYIILQLPAPDFR

SEQ ID NO: 10 - protein, 450 aa, synthetic construct
EVQLVESGGGLVQPGGSLRLSCAASGIDLSNYAMGWVRQAPGKGLEWVGYISGGGSAYYASWAKGRFTISRDNSKNTLYLQMNSLRAEDTAVYYCARWAIKSYFFGMDLWGQGTLVTVSSASTKGPSVFPLAPSSKSTSGGTAALGCLVKDYFPEPVTVSWNSGALTSGVHTFPAVLQSSGLYSLSSVVTVPSSSLGTQTYICNVNHKPSNTKVDKRVEPKSCDKTHTCPPCPAPEAAGGPSVFLFPPKPKDTLMISRTPEVTCVVVDVSHEDPEVKFNWYVDGVEVHNAKTKPREEQYNSTYRVVSVLTVLHQDWLNGKEYKCKVSNKALPAPIEKTISKAKGQPREPQVYTLPPSREEMTKNQVSLTCLVKGFYPSDIAVEWESNGQPENNYKTTPPVLDSDGSFFLYSKLTVDKSRWQQGNVFSCSVMHEALHNHYTQKSLSLSPGK

SEQ ID NO: 11 - protein, 217 aa, synthetic construct
DIQMTQSPSSVSASVGDRVTITCQASEYISSYLAWYQQKPGKAPKLLIYQASTLASGVPSRFSGSGSGTDFTLTISSLQPEDFATYYCQTNNAIHTYGGAFGGGTKVEIKRTVAAPSVFIFPPSDEQLKSGTASVVCLLNNFYPREAKVQWKVDNALQSGNSQESVTEQDSKDSTYSLSSTLTLSKADYEKHKVYACEVTHQGLSSPVTKSFNRGEC